European Patent Specification EP 3 310 814 B1, published August 2, 2023. Title: HUMANIZED AND AFFINITY MATURED ANTIBODIES TO FcRH5 AND METHODS OF USE. Applicant: Genentech, Inc. F. Hoffmann-La Roche AG. The sequence listing filed with the application follows.

SEQUENCE LISTING (215 sequences)

SEQ ID NO: 1 - protein, 5 aa, Artificial Sequence
  Synthetic construct
RFGVH

SEQ ID NO: 2 - protein, 16 aa, Artificial Sequence
  Synthetic construct
  MISC_FEATURE (12)..(12): Xaa is Ala or Pro
  MISC_FEATURE (15)..(15): Xaa is Met, Gly, or Val
  MISC_FEATURE (16)..(16): Xaa is Ser, Asp, or Pro
VIWRGGSTDYNXAFXX

SEQ ID NO: 3 - protein, 12 aa, Artificial Sequence
  Synthetic construct
  MISC_FEATURE (6)..(6): Xaa is Ser or Pro
HYYGSXDYALDN

SEQ ID NO: 4 - protein, 11 aa, Artificial Sequence
  Synthetic construct
  MISC_FEATURE (7)..(7): Xaa is Ser or Arg
  MISC_FEATURE (9)..(9): Xaa is Ile or Leu
KASQDVXNXVV

SEQ ID NO: 5 - protein, 7 aa, Artificial Sequence
  Synthetic construct
  MISC_FEATURE (2)..(2): Xaa is Ala or Gly
  MISC_FEATURE (3)..(3): Xaa is Ser or Tyr
  MISC_FEATURE (4)..(4): Xaa is Tyr or Asn
  MISC_FEATURE (7)..(7): Xaa is Thr or Ser
SXXXRYX

SEQ ID NO: 6 - protein, 9 aa, Artificial Sequence
  Synthetic construct
  MISC_FEATURE (3)..(3): Xaa is His or Gln
  MISC_FEATURE (4)..(4): Xaa is Tyr or Phe
  MISC_FEATURE (5)..(5): Xaa is Gln or Ser
  MISC_FEATURE (6)..(6): Xaa is Ser or Pro
QQXXXXPYT

SEQ ID NO: 7 - protein, 16 aa, Artificial Sequence
  Synthetic construct
VIWRGGSTDYNAAFMS

SEQ ID NO: 8 - protein, 16 aa, Artificial Sequence
  Synthetic construct
VIWRGGSTDYNAAFVS

SEQ ID NO: 9 - protein, 12 aa, Artificial Sequence
  Synthetic construct
HYYGSSDYALDN

SEQ ID NO: 10 - protein, 12 aa, Artificial Sequence
  Synthetic construct
HYYGSPDYALDN

SEQ ID NO: 11 - protein, 11 aa, Artificial Sequence
  Synthetic construct
KASQDVSNIVV

SEQ ID NO: 12 - protein, 11 aa, Artificial Sequence
  Synthetic construct
KASQDVRNLVV

SEQ ID NO: 13 - protein, 11 aa, Artificial Sequence
  Synthetic construct
KASQDVRNIVV

SEQ ID NO: 14 - protein, 11 aa, Artificial Sequence
  Synthetic construct
KASQDVSNLVV

SEQ ID NO: 15 - protein, 7 aa, Artificial Sequence
  Synthetic construct
SASYRYT

SEQ ID NO: 16 - protein, 7 aa, Artificial Sequence
  Synthetic construct
SGSYRYS

SEQ ID NO: 17 - protein, 7 aa, Artificial Sequence
  Synthetic construct
SGYNRYS

SEQ ID NO: 18 - protein, 7 aa, Artificial Sequence
  Synthetic construct
SGYYRYT

SEQ ID NO: 19 - protein, 7 aa, Artificial Sequence
  Synthetic construct
SGYYRYS

SEQ ID NO: 20 - protein, 9 aa, Artificial Sequence
  Synthetic construct
QQHYSSPYT

SEQ ID NO: 21 - protein, 9 aa, Artificial Sequence
  Synthetic construct
QQQYSPPYT

SEQ ID NO: 22 - protein, 9 aa, Artificial Sequence
  Synthetic construct
QQQFQPPYT

SEQ ID NO: 23 - protein, 9 aa, Artificial Sequence
  Synthetic construct
QQHYSPPYT

SEQ ID NO: 24 - protein, 9 aa, Artificial Sequence
  Synthetic construct
QQQYQPPYT

SEQ ID NO: 25 - protein, 9 aa, Artificial Sequence
  Synthetic construct
QQHYQPPYT

SEQ ID NO: 26 - protein, 10 aa, Artificial Sequence
  Synthetic construct
GIDLSSYAMG

SEQ ID NO: 27 - protein, 16 aa, Artificial Sequence
  Synthetic construct
TIGTGGTPYYASWAKG

SEQ ID NO: 28 - protein, 13 aa, Artificial Sequence
  Synthetic construct
ARDMYTGSIYYDM

SEQ ID NO: 29 - protein, 13 aa, Artificial Sequence
  Synthetic construct
QSSQSVFNNAQLS

SEQ ID NO: 30 - protein, 7 aa, Artificial Sequence
  Synthetic construct
DTSNLAS

SEQ ID NO: 31 - protein, 11 aa, Artificial Sequence
  Synthetic construct
LGAYTDDADNA

SEQ ID NO: 32 - protein, 10 aa, Artificial Sequence
  Synthetic construct
GYTFTHYAMH

SEQ ID NO: 33 - protein, 17 aa, Artificial Sequence
  Synthetic construct
MISSSSGNTNFNQKFMD

SEQ ID NO: 34 - protein, 11 aa, Artificial Sequence
  Synthetic construct
ARWSYYALFDY

SEQ ID NO: 35 - protein, 10 aa, Artificial Sequence
  Synthetic construct
SADSSVDYIH

SEQ ID NO: 36 - protein, 7 aa, Artificial Sequence
  Synthetic construct
DTSKLAS

SEQ ID NO: 37 - protein, 9 aa, Artificial Sequence
  Synthetic construct
FQGSGYPLT

SEQ ID NO: 38 - protein, 10 aa, Artificial Sequence
  Synthetic construct
GYTFTNYVIH

SEQ ID NO: 39 - protein, 17 aa, Artificial Sequence
  Synthetic construct
YISPYNDYTKYNEKFEG

SEQ ID NO: 40 - protein, 11 aa, Artificial Sequence
  Synthetic construct
ARRDYYGSSDY

SEQ ID NO: 41 - protein, 10 aa, Artificial Sequence
  Synthetic construct
SASSSVDYMH

SEQ ID NO: 42 - protein, 7 aa, Artificial Sequence
  Synthetic construct
DTSKLAS

SEQ ID NO: 43 - protein, 9 aa, Artificial Sequence
  Synthetic construct
QQWSSNPPT

SEQ ID NO: 44 - protein, 30 aa, Artificial Sequence
  Synthetic construct
  MISC_FEATURE (1)..(1): Xaa is Glu, Ser, or Phe
  MISC_FEATURE (28)..(28): Xaa is Ser or Pro
  MISC_FEATURE (29)..(29): Xaa is Leu or Thr
XVQLVESGPGLVKPSETLSLTCTVSGFXXT

SEQ ID NO: 45 - protein, 14 aa, Artificial Sequence
  Synthetic construct
  MISC_FEATURE (2)..(2): Xaa is Val or Tyr
  MISC_FEATURE (13)..(13): Xaa is Leu or Ile
WXRQPPGKGLEWXG

SEQ ID NO: 46 - protein, 32 aa, Artificial Sequence
  Synthetic construct
RLTISKDNSKNQVSLKLSSVTAADTAVYYCSN

SEQ ID NO: 47 - protein, 11 aa, Artificial Sequence
  Synthetic construct
WGQGTLVTVSS

SEQ ID NO: 48 - protein, 23 aa, Artificial Sequence
  Synthetic construct
DIQMTQSPSSLSASVGDRVTITC

SEQ ID NO: 49 - protein, 15 aa, Artificial Sequence
  Synthetic construct
  MISC_FEATURE (9)..(9): Xaa is Ala or Ser
WFQQKPGKXPKLLIY

SEQ ID NO: 50 - protein, 32 aa, Artificial Sequence
  Synthetic construct
GVPSRFSGSGSGTDFTLTISSLQPEDFATYYC

SEQ ID NO: 51 - protein, 10 aa, Artificial Sequence
  Synthetic construct
FGQGTKVEIK

SEQ ID NO: 52 - protein, 30 aa, Artificial Sequence
  Synthetic construct
EVQLVESGPGLVKPSETLSLTCTVSGFSLT

SEQ ID NO: 53 - protein, 30 aa, Artificial Sequence
  Synthetic construct
EVQLVESGPGLVKPSETLSLTCTVSGFSTT

SEQ ID NO: 54 - protein, 14 aa, Artificial Sequence
  Synthetic construct
WVRQPPGKGLEWLG

SEQ ID NO: 55 - protein, 14 aa, Artificial Sequence
  Synthetic construct
WVRQPPGKGLEWIG

SEQ ID NO: 56 - protein, 15 aa, Artificial Sequence
  Synthetic construct
WFQQKPGKSPKLLIY

SEQ ID NO: 57 - protein, 15 aa, Artificial Sequence
  Synthetic construct
WFQQKPGKAPKLLIY

SEQ ID NO: 58 - protein, 25 aa, Artificial Sequence [sequence omitted]

SEQ ID NO: 59 - protein, 14 aa, Artificial Sequence
  Synthetic construct
WVRQAPGKGLEWIG

SEQ ID NO: 60 - protein, 30 aa, Artificial Sequence
  Synthetic construct
RFTISKDSSKNTVYLQMNSLRAEDTAVYFC

SEQ ID NO: 61 - protein, 11 aa, Artificial Sequence
  Synthetic construct
WGQGTLVTVSS

SEQ ID NO: 62 - protein, 22 aa, Artificial Sequence
  Synthetic construct
DAQLTQSPSSLSASVGDRVTIT

SEQ ID NO: 63 - protein, 15 aa, Artificial Sequence
  Synthetic construct
WYQQKPGKPPKLLIY

SEQ ID NO: 64 - protein, 32 aa, Artificial Sequence; identical to SEQ ID NO: 50
  Synthetic construct

SEQ ID NO: 65 - protein, 10 aa, Artificial Sequence
  Synthetic construct
FGQGTKVEIK

SEQ ID NO: 66 - protein, 25 aa, Artificial Sequence
  Synthetic construct
QVQLQQSGPELVRPGVSVKISCKGS

SEQ ID NO: 67 - protein, 14 aa, Artificial Sequence
  Synthetic construct
WVKQSHTKSLEWIG

SEQ ID NO: 68 - protein, 30 aa, Artificial Sequence
  Synthetic construct
KATMTVDKSSTTAYLELARLTFGDSAIYYC

SEQ ID NO: 69 - protein, 11 aa, Artificial Sequence
  Synthetic construct
WGQGTTVTVSS

SEQ ID NO: 70 - protein, 23 aa, Artificial Sequence
  Synthetic construct
ENVLTQSPAIMSASPGEKVTMTC

SEQ ID NO: 71 - protein, 15 aa, Artificial Sequence
  Synthetic construct
WYQQKSNTSPKLWIY

SEQ ID NO: 72 - protein, 32 aa, Artificial Sequence
  Synthetic construct
GVPGRFSGSGSGNSYSLTISSMEAEDFATYYC

SEQ ID NO: 73 - protein, 10 aa, Artificial Sequence
  Synthetic construct
FGSGTKLELK

SEQ ID NO: 74 - protein, 25 aa, Artificial Sequence
  Synthetic construct
EVQLQQSGPELVKPGASVKMSCKAS

SEQ ID NO: 75 - protein, 14 aa, Artificial Sequence
  Synthetic construct
WMKQKPGQGLEWIG

SEQ ID NO: 76 - protein, 30 aa, Artificial Sequence
  Synthetic construct
KATLTSDKSSNTAYMELSSLTSEDSAVYYC

SEQ ID NO: 77 - protein, 11 aa, Artificial Sequence
  Synthetic construct
WGQGTTLTVSS

SEQ ID NO: 78 - protein, 23 aa, Artificial Sequence
  Synthetic construct
QIVLTQSPAIMSASPGEKVTMTC

SEQ ID NO: 79 - protein, 15 aa, Artificial Sequence
  Synthetic construct
WYQQKSGTSPKKWIY

SEQ ID NO: 80 - protein, 32 aa, Artificial Sequence
  Synthetic construct
GVPARFSGSGSGTSYSLTIGSMEAEDAATYYC

SEQ ID NO: 81 - protein, 10 aa, Artificial Sequence
  Synthetic construct
FGGGTKLEIK

SEQ ID NO: 82 - protein, 120 aa, Artificial Sequence
  Synthetic construct
EVQLVESGPGLVKPSETLSLTCTVSGFSLTRFGVHWVRQPPGKGLEWLGVIWRGGSTDYNAAFMSRLTISKDNSKNQVSLKLSSVTAADTAVYYCSNHYYGSSDYALDNWGQGTLVTVSS

SEQ ID NO: 83 - protein, 107 aa, Artificial Sequence
  Synthetic construct
DIQMTQSPSSLSASVGDRVTITCKASQDVSNIVVWFQQKPGKSPKLLIYSASYRYTGVPSRFSGSGSGTDFTLTISSLQPEDFATYYCQQHYSSPYTFGQGTKVEIK

SEQ ID NO: 84 - protein, 120 aa, Artificial Sequence; identical to SEQ ID NO: 82
  Synthetic construct

SEQ ID NO: 85 - protein, 107 aa, Artificial Sequence
  Synthetic construct
DIQMTQSPSSLSASVGDRVTITCKASQDVRNLVVWFQQKPGKAPKLLIYSGSYRYSGVPSRFSGSGSGTDFTLTISSLQPEDFATYYCQQQYSPPYTFGQGTKVEIK

SEQ ID NO: 86 - protein, 120 aa, Artificial Sequence; identical to SEQ ID NO: 82
  Synthetic construct

SEQ ID NO: 87 - protein, 107 aa, Artificial Sequence
  Synthetic construct
DIQMTQSPSSLSASVGDRVTITCKASQDVRNLVVWFQQKPGKAPKLLIYSGYNRYSGVPSRFSGSGSGTDFTLTISSLQPEDFATYYCQQQFQPPYTFGQGTKVEIK

SEQ ID NO: 88 - protein, 120 aa, Artificial Sequence; identical to SEQ ID NO: 82
  Synthetic construct

SEQ ID NO: 89 - protein, 107 aa, Artificial Sequence
  Synthetic construct
DIQMTQSPSSLSASVGDRVTITCKASQDVRNIVVWFQQKPGKAPKLLIYSGSYRYSGVPSRFSGSGSGTDFTLTISSLQPEDFATYYCQQQYSPPYTFGQGTKVEIK

SEQ ID NO: 90 - protein, 120 aa, Artificial Sequence; identical to SEQ ID NO: 82
  Synthetic construct

SEQ ID NO: 91 - protein, 107 aa, Artificial Sequence
  Synthetic construct
DIQMTQSPSSLSASVGDRVTITCKASQDVRNLVVWFQQKPGKAPKLLIYSGSYRYSGVPSRFSGSGSGTDFTLTISSLQPEDFATYYCQQHYSPPYTFGQGTKVEIK

SEQ ID NO: 92 - protein, 120 aa, Artificial Sequence; identical to SEQ ID NO: 82
  Synthetic construct

SEQ ID NO: 93 - protein, 107 aa, Artificial Sequence
  Synthetic construct
DIQMTQSPSSLSASVGDRVTITCKASQDVSNIVVWFQQKPGKSPKLLIYSGYYRYTGVPSRFSGSGSGTDFTLTISSLQPEDFATYYCQQQFQPPYTFGQGTKVEIK

SEQ ID NO: 94 - protein, 120 aa, Artificial Sequence; identical to SEQ ID NO: 82
  Synthetic construct

SEQ ID NO: 95 - protein, 107 aa, Artificial Sequence
  Synthetic construct
DIQMTQSPSSLSASVGDRVTITCKASQDVSNIVVWFQQKPGKAPKLLIYSGYYRYSGVPSRFSGSGSGTDFTLTISSLQPEDFATYYCQQQYQPPYTFGQGTKVEIK

SEQ ID NO: 96 - protein, 120 aa, Artificial Sequence
  Synthetic construct
EVQLVESGPGLVKPSETLSLTCTVSGFSTTRFGVHWVRQPPGKGLEWLGVIWRGGSTDYNAAFMSRLTISKDNSKNQVSLKLSSVTAADTAVYYCSNHYYGSSDYALDNWGQGTLVTVSS

SEQ ID NO: 97 - protein, 107 aa, Artificial Sequence
  Synthetic construct
DIQMTQSPSSLSASVGDRVTITCKASQDVRNLVVWFQQKPGKAPKLLIYSGYYRYTGVPSRFSGSGSGTDFTLTISSLQPEDFATYYCQQHYQPPYTFGQGTKVEIK

SEQ ID NO: 98 - protein, 120 aa, Artificial Sequence
  Synthetic construct
EVQLVESGPGLVKPSETLSLTCTVSGFSLTRFGVHWVRQPPGKGLEWIGVIWRGGSTDYNAAFMSRLTISKDNSKNQVSLKLSSVTAADTAVYYCSNHYYGSSDYALDNWGQGTLVTVSS

SEQ ID NO: 99 - protein, 107 aa, Artificial Sequence; identical to SEQ ID NO: 97
  Synthetic construct

SEQ ID NO: 100 - protein, 120 aa, Artificial Sequence; identical to SEQ ID NO: 82
  Synthetic construct

SEQ ID NO: 101 - protein, 107 aa, Artificial Sequence; identical to SEQ ID NO: 97
  Synthetic construct

SEQ ID NO: 102 - protein, 120 aa, Artificial Sequence
  Synthetic construct
EVQLVESGPGLVKPSETLSLTCTVSGFSLTRFGVHWVRQPPGKGLEWLGVIWRGGSTDYNAAFVSRLTISKDNSKNQVSLKLSSVTAADTAVYYCSNHYYGSSDYALDNWGQGTLVTVSS

SEQ ID NO: 103 - protein, 107 aa, Artificial Sequence; identical to SEQ ID NO: 83
  Synthetic construct

SEQ ID NO: 104 - protein, 120 aa, Artificial Sequence; identical to SEQ ID NO: 102
  Synthetic construct

SEQ ID NO: 105 - protein, 107 aa, Artificial Sequence; identical to SEQ ID NO: 91
  Synthetic construct

SEQ ID NO: 106 - protein, 120 aa, Artificial Sequence
  Synthetic construct
EVQLVESGPGLVKPSETLSLTCTVSGFSTTRFGVHWVRQPPGKGLEWLGVIWRGGSTDYNAAFVSRLTISKDNSKNQVSLKLSSVTAADTAVYYCSNHYYGSPDYALDNWGQGTLVTVSS

SEQ ID NO: 107 - protein, 107 aa, Artificial Sequence
  Synthetic construct
DIQMTQSPSSLSASVGDRVTITCKASQDVSNLVVWFQQKPGKAPKLLIYSGSYRYSGVPSRFSGSGSGTDFTLTISSLQPEDFATYYCQQHYSPPYTFGQGTKVEIK

SEQ ID NO: 108 - protein, 119 aa, Artificial Sequence
  Synthetic construct
EVQLVESGGGLVQPGGSLRLSCAVSGIDLSSYAMGWVRQAPGKGLEWIGTIGTGGTPYYASWAKGRFTISKDSSKNTVYLQMNSLRAEDTAVYFCARDMYTGSIYYDMWGQGTLVTVSS

SEQ ID NO: 109 - protein, 111 aa, Artificial Sequence
  Synthetic construct
DAQLTQSPSSLSASVGDRVTITCQSSQSVFNNAQLSWYQQKPGKPPKLLIYDTSNLASGVPSRFSGSGSGTDFTLTISSLQPEDFATYYCLGAYTDDADNAFGQGTKVEIK

SEQ ID NO: 110 - protein, 118 aa, Artificial Sequence
  Synthetic construct
QVQLQQSGPELVRPGVSVKISCKGSGYTFTHYAMHWVKQSHTKSLEWIGMISSSSGNTNFNQKFMDKATMTVDKSSTTAYLELARLTFGDSAIYYCARWSYYALFDYWGQGTTVTVSS

SEQ ID NO: 111 - protein, 106 aa, Artificial Sequence
  Synthetic construct
ENVLTQSPAIMSASPGEKVTMTCSADSSVDYIHWYQQKSNTSPKLWIYDTSKLASGVPGRFSGSGSGNSYSLTISSMEAEDFATYYCFQGSGYPLTFGSGTKLELK

SEQ ID NO: 112 - protein, 118 aa, Artificial Sequence
  Synthetic construct
EVQLQQSGPELVKPGASVKMSCKASGYTFTNYVIHWMKQKPGQGLEWIGYISPYNDYTKYNEKFEGKATLTSDKSSNTAYMELSSLTSEDSAVYYCARRDYYGSSDYWGQGTTLTVSS

SEQ ID NO: 113 - protein, 106 aa, Artificial Sequence
  Synthetic construct
QIVLTQSPAIMSASPGEKVTMTCSASSSVDYMHWYQQKSGTSPKKWIYDTSKLASGVPARFSGSGSGTSYSLTIGSMEAEDAATYYCQQWSSNPPTFGGGTKLEIK

SEQ ID NO: 114 - protein, 977 aa, Homo sapiens
MLLWVILLVLAPVSGQFARTPRPIIFLQPPWTTVFQGERVTLTCKGFRFYSPQKTKWYHRYLGKEILRETPDNILEVQESGEYRCQAQGSPLSSPVHLDFSSASLILQAPLSVFEGDSVVLRCRAKAEVTLNNTIYKNDNVLAFLNKRTDFHIPHACLKDNGAYRCTGYKESCCPVSSNTVKIQVQEPFTRPVLRASSFQPISGNPVTLTCETQLSLERSDVPLRFRFFRDDQTLGLGWSLSPNFQITAMWSKDSGFYWCKAATMPYSVISDSPRSWIQVQIPASHPVLTLSPEKALNFEGTKVTLHCETQEDSLRTLYRFYHEGVPLRHKSVRCERGASISFSLTTENSGNYYCTADNGLGAKPSKAVSLSVTVPVSHPVLNLSSPEDLIFEGAKVTLHCEAQRGSLPILYQFHHEGAALERRSANSAGGVAISFSLTAEHSGNYYCTADNGFGPQRSKAVSLSVTVPVSHPVLTLSSAEALTFEGATVTLHCEVQRGSPQILYQFYHEDMPLWSSSTPSVGRVSFSFSLTEGHSGNYYCTADNGFGPQRSEVVSLFVTVPVSRPILTLRVPRAQAVVGDLLELHCEAPRGSPPILYWFYHEDVTLGSSSAPSGGEASFNLSLTAEHSGNYSCEANNGLVAQHSDTISLSVIVPVSRPILTFRAPRAQAVVGDLLELHCEALRGSSPILYWFYHEDVTLGKISAPSGGGASFNLSLTTEHSGIYSCEADNGLEAQRSEMVTLKVAVPVSRPVLTLRAPGTHAAVGDLLELHCEALRGSPLILYRFFHEDVTLGNRSSPSGGASLNLSLTAEHSGNYSCEADNGLGAQRSETVTLYITGLTANRSGPFATGVAGGLLSIAGLAAGALLLYCWLSRKAGRKPASDPARSPSDSDSQEPTYHNVPAWEELQPVYTNANPRGENVVYSEVRIIQEKKKHAVASDPRHLRNKGSPIIYSEVKVASTPVSGSLFLASSAPHR

SEQ ID NO: 115 - protein, 5 aa, Artificial Sequence
  Synthetic construct
SYYIH

SEQ ID NO: 116 - protein, 17 aa, Artificial Sequence
  Synthetic construct
WIYPENDNTKYNEKFKD

SEQ ID NO: 117 - protein, 10 aa, Artificial Sequence
  Synthetic construct
  MISC_FEATURE (6)..(6): Xaa is Tyr or Ala
DGYSRXYFDY

SEQ ID NO: 118 - protein, 17 aa, Artificial Sequence
  Synthetic construct
KSSQSLLNSRTRKNYLA

SEQ ID NO: 119 - protein, 7 aa, Artificial Sequence
  Synthetic construct
WTSTRKS

SEQ ID NO: 120 - protein, 8 aa, Artificial Sequence
  Synthetic construct
  MISC_FEATURE (1)..(1): Xaa is Lys or Thr
XQSFILRT

SEQ ID NO: 121 - protein, 10 aa, Artificial Sequence
  Synthetic construct
DGYSRYYFDY

SEQ ID NO: 122 - protein, 10 aa, Artificial Sequence
  Synthetic construct
DGYSRAYFDY

SEQ ID NO: 123 - protein, 8 aa, Artificial Sequence
  Synthetic construct
KQSFILRT

SEQ ID NO: 124 - protein, 8 aa, Artificial Sequence
  Synthetic construct
TQSFILRT

SEQ ID NO: 125 - protein, 30 aa, Artificial Sequence
  Synthetic construct
EVQLVQSGAEVKKPGASVKVSCKASGFTFT

SEQ ID NO: 126 - protein, 14 aa, Artificial Sequence
  Synthetic construct
WVRQAPGQGLEWIG

SEQ ID NO: 127 - protein, 32 aa, Artificial Sequence
  Synthetic construct
RVTITADTSTSTAYLELSSLRSEDTAVYYCAR

SEQ ID NO: 128 - protein, 11 aa, Artificial Sequence
  Synthetic construct
WGQGTLVTVSS

SEQ ID NO: 129 - protein, 23 aa, Artificial Sequence
  Synthetic construct
DIVMTQSPDSLAVSLGERATINC

SEQ ID NO: 130 - protein, 15 aa, Artificial Sequence
  Synthetic construct
WYQQKPGQSPKLLIY

SEQ ID NO: 131 - protein, 32 aa, Artificial Sequence
  Synthetic construct
GVPDRFSGSGSGTDFTLTISSLQAEDVAVYYC

SEQ ID NO: 132 - protein, 10 aa, Artificial Sequence
  Synthetic construct
FGQGTKVEIK

SEQ ID NO: 133 - protein, 119 aa, Artificial Sequence
  Synthetic construct
EVQLVQSGAEVKKPGASVKVSCKASGFTFTSYYIHWVRQAPGQGLEWIGWIYPENDNTKYNEKFKDRVTITADTSTSTAYLELSSLRSEDTAVYYCARDGYSRYYFDYWGQGTLVTVSS

SEQ ID NO: 134 - protein, 112 aa, Artificial Sequence
  Synthetic construct
DIVMTQSPDSLAVSLGERATINCKSSQSLLNSRTRKNYLAWYQQKPGQSPKLLIYWTSTRKSGVPDRFSGSGSGTDFTLTISSLQAEDVAVYYCKQSFILRTFGQGTKVEIK

SEQ ID NO: 135 - protein, 119 aa, Artificial Sequence
  Synthetic construct
EVQLVQSGAEVKKPGASVKVSCKASGFTFTSYYIHWVRQAPGQGLEWIGWIYPENDNTKYNEKFKDRVTITADTSTSTAYLELSSLRSEDTAVYYCARDGYSRAYFDYWGQGTLVTVSS

SEQ ID NO: 136 - protein, 112 aa, Artificial Sequence; identical to SEQ ID NO: 134
  Synthetic construct

SEQ ID NO: 137 - protein, 119 aa, Artificial Sequence; identical to SEQ ID NO: 133
  Synthetic construct

SEQ ID NO: 138 - protein, 112 aa, Artificial Sequence
  Synthetic construct
DIVMTQSPDSLAVSLGERATINCKSSQSLLNSRTRKNYLAWYQQKPGQSPKLLIYWTSTRKSGVPDRFSGSGSGTDFTLTISSLQAEDVAVYYCTQSFILRTFGQGTKVEIK

SEQ ID NO: 139 - protein, 5 aa, Artificial Sequence
  Synthetic construct
NYYIH

SEQ ID NO: 140 - protein, 17 aa, Artificial Sequence
  Synthetic construct
WIYPGDGNTKYNEKFKG

SEQ ID NO: 141 - protein, 10 aa, Artificial Sequence
  Synthetic construct
DSYSNYYFDY

SEQ ID NO: 142 - protein, 17 aa, Artificial Sequence
  Synthetic construct
KSSQSLLNSRTRKNYLA

SEQ ID NO: 143 - protein, 7 aa, Artificial Sequence
  Synthetic construct
WASTRES

SEQ ID NO: 144 - protein, 8 aa, Artificial Sequence
  Synthetic construct
TQSFILRT

SEQ ID NO: 145 - protein, 30 aa, Artificial Sequence
  Synthetic construct
EVQLVQSGAEVKKPGASVKVSCKASGYTFT

SEQ ID NO: 146 - protein, 14 aa, Artificial Sequence
  Synthetic construct
WVRQAPGQGLEWIG

SEQ ID NO: 147 - protein, 32 aa, Artificial Sequence
  Synthetic construct
RATLTADTSTSTAYLELSSLRSEDTAVYYCAR

SEQ ID NO: 148 - protein, 11 aa, Artificial Sequence
  Synthetic construct
WGQGTLVTVSS

SEQ ID NO: 149 - protein, 23 aa, Artificial Sequence
  Synthetic construct
DIVMTQSPDSLAVSLGERATINC

SEQ ID NO: 150 - protein, 15 aa, Artificial Sequence
  Synthetic construct
WYQQKPGQPPKLLIY

SEQ ID NO: 151 - protein, 32 aa, Artificial Sequence; identical to SEQ ID NO: 131
  Synthetic construct

SEQ ID NO: 152 - protein, 10 aa, Artificial Sequence
  Synthetic construct
FGQGTKVEIK

SEQ ID NO: 153 - protein, 119 aa, Artificial Sequence
  Synthetic construct
EVQLVQSGAEVKKPGASVKVSCKASGYTFTNYYIHWVRQAPGQGLEWIGWIYPGDGNTKYNEKFKGRATLTADTSTSTAYLELSSLRSEDTAVYYCARDSYSNYYFDYWGQGTLVTVSS

SEQ ID NO: 154 - protein, 112 aa, Artificial Sequence
  Synthetic construct
DIVMTQSPDSLAVSLGERATINCKSSQSLLNSRTRKNYLAWYQQKPGQPPKLLIYWASTRESGVPDRFSGSGSGTDFTLTISSLQAEDVAVYYCTQSFILRTFGQGTKVEIK

SEQ ID NO: 155 - protein, 5 aa, Artificial Sequence
  Synthetic construct
GYTMN

SEQ ID NO: 156 - protein, 17 aa, Artificial Sequence
  Synthetic construct
  MISC_FEATURE (9)..(9): Xaa is Ser or Thr
  MISC_FEATURE (12)..(12): Xaa is Asn or Ala
  MISC_FEATURE (13)..(13): Xaa is Gln or Asp
  MISC_FEATURE (14)..(14): Xaa is Lys or Ser
  MISC_FEATURE (15)..(15): Xaa is Val or Phe
  MISC_FEATURE (17)..(17): Xaa is Gly or Asp
LINPYKGVXTYXXXXKX

SEQ ID NO: 157 - protein, 13 aa, Artificial Sequence
  Synthetic construct
SGYYGDSDWYFDV

SEQ ID NO: 158 - protein, 11 aa, Artificial Sequence
  Synthetic construct
RASQDIRNYLN

SEQ ID NO: 159 - protein, 7 aa, Artificial Sequence
  Synthetic construct
YTSRLES

SEQ ID NO: 160 - protein, 9 aa, Artificial Sequence
  Synthetic construct
QQGNTLPWT

SEQ ID NO: 161 - protein, 17 aa, Artificial Sequence
  Synthetic construct
LINPYKGVTTYADSVKG

SEQ ID NO: 162 - protein, 17 aa, Artificial Sequence
  Synthetic construct
LINPYKGVSTYNQKFKD

SEQ ID NO: 163 - protein, 17 aa, Artificial Sequence
  Synthetic construct
LINPYKGVSTYADSVKG

SEQ ID NO: 164 - protein, 30 aa, Artificial Sequence
  Synthetic construct
EVQLVESGGGLVQPGGSLRLSCAASGYSFT

SEQ ID NO: 165 - protein, 14 aa, Artificial Sequence
  Synthetic construct
WVRQAPGKDLEWVA

SEQ ID NO: 166 - protein, 32 aa, Artificial Sequence
  Synthetic construct
RFTISVDKSKNTAYLQMNSLRAEDTAVYYCAR

SEQ ID NO: 167 - protein, 11 aa, Artificial Sequence
  Synthetic construct
WGQGTLVTVSS

SEQ ID NO: 168 - protein, 23 aa, Artificial Sequence
  Synthetic construct
DIQMTQSPSSLSASVGDRVTITC

SEQ ID NO: 169 - protein, 15 aa, Artificial Sequence
  Synthetic construct
WYQQKPGKAPKLLIY

SEQ ID NO: 170 - protein, 32 aa, Artificial Sequence
  Synthetic construct
GVPSRFSGSGSGTDYTLTISSLQPEDFATYYC

SEQ ID NO: 171 - protein, 10 aa, Artificial Sequence
  Synthetic construct
FGQGTKLELK

SEQ ID NO: 172 - protein, 122 aa, Artificial Sequence
  Synthetic construct
EVQLVESGGGLVQPGGSLRLSCAASGYSFTGYTMNWVRQAPGKDLEWVALINPYKGVSTYNQKFKDRFTISVDKSKNTAYLQMNSLRAEDTAVYYCARSGYYGDSDWYFDVWGQGTLVTVSS

SEQ ID NO: 173 - protein, 107 aa, Artificial Sequence
  Synthetic construct
DIQMTQSPSSLSASVGDRVTITCRASQDIRNYLNWYQQKPGKAPKLLIYYTSRLESGVPSRFSGSGSGTDYTLTISSLQPEDFATYYCQQGNTLPWTFGQGTKLELK

SEQ ID NO: 174 - protein, 28 aa, Artificial Sequence
  Synthetic construct
QDGNEEMGGITQTPYKVSISGTTVILTC

SEQ ID NO: 175 - protein, 16 aa, Artificial Sequence
  Synthetic construct
VIWRGGSTDYNPAFMS

SEQ ID NO: 176 - protein, 16 aa, Artificial Sequence
  Synthetic construct
VIWRGGSTDYNAAFGS

SEQ ID NO: 177 - protein, 16 aa, Artificial Sequence
  Synthetic construct
VIWRGGSTDYNAAFMD

SEQ ID NO: 178 - protein, 16 aa, Artificial Sequence
  Synthetic construct
VIWRGGSTDYNAAFMP

SEQ ID NO: 179 - protein, 30 aa, Artificial Sequence
  Synthetic construct
SVQLVESGPGLVKPSETLSLTCTVSGFSLT

SEQ ID NO: 180 - protein, 30 aa, Artificial Sequence
  Synthetic construct
FVQLVESGPGLVKPSETLSLTCTVSGFSLT

SEQ ID NO: 181 - protein, 30 aa, Artificial Sequence
  Synthetic construct
EVQLVESGPGLVKPSETLSLTCTVSGFPLT

SEQ ID NO: 182 - protein, 14 aa, Artificial Sequence
  Synthetic construct
WYRQPPGKGLEWLG

SEQ ID NO: 183 - protein, 32 aa, Artificial Sequence
  Synthetic construct
RLTISKDNSKNQVSLMLSSVTAADTAVYYCSN

SEQ ID NO: 184 - protein, 32 aa, Artificial Sequence
  Synthetic construct
RLTISKDNSKNQVSLKLSDVTAADTAVYYCSN

SEQ ID NO: 185 - protein, 120 aa, Artificial Sequence
  Synthetic construct
SVQLVESGPGLVKPSETLSLTCTVSGFSLTRFGVHWVRQPPGKGLEWLGVIWRGGSTDYNAAFMSRLTISKDNSKNQVSLKLSSVTAADTAVYYCSNHYYGSSDYALDNWGQGTLVTVSS

SEQ ID NO: 186 - protein, 107 aa, Artificial Sequence; identical to SEQ ID NO: 83
  Synthetic construct

SEQ ID NO: 187 - protein, 120 aa, Artificial Sequence
  Synthetic construct
FVQLVESGPGLVKPSETLSLTCTVSGFSLTRFGVHWVRQPPGKGLEWLGVIWRGGSTDYNAAFMSRLTISKDNSKNQVSLKLSSVTAADTAVYYCSNHYYGSSDYALDNWGQGTLVTVSS

SEQ ID NO: 188 - protein, 107 aa, Artificial Sequence; identical to SEQ ID NO: 83
  Synthetic construct

SEQ ID NO: 189 - protein, 120 aa, Artificial Sequence
  Synthetic construct
EVQLVESGPGLVKPSETLSLTCTVSGFPLTRFGVHWVRQPPGKGLEWLGVIWRGGSTDYNAAFMSRLTISKDNSKNQVSLKLSSVTAADTAVYYCSNHYYGSSDYALDNWGQGTLVTVSS

SEQ ID NO: 190 - protein, 107 aa, Artificial Sequence; identical to SEQ ID NO: 83
  Synthetic construct

SEQ ID NO: 191 - protein, 120 aa, Artificial Sequence; identical to SEQ ID NO: 96
  Synthetic construct

SEQ ID NO: 192 - protein, 107 aa, Artificial Sequence; identical to SEQ ID NO: 83
  Synthetic construct

SEQ ID NO: 193 - protein, 120 aa, Artificial Sequence
  Synthetic construct
EVQLVESGPGLVKPSETLSLTCTVSGFSLTRFGVHWYRQPPGKGLEWLGVIWRGGSTDYNAAFMSRLTISKDNSKNQVSLKLSSVTAADTAVYYCSNHYYGSSDYALDNWGQGTLVTVSS

SEQ ID NO: 194 - protein, 107 aa, Artificial Sequence; identical to SEQ ID NO: 83
  Synthetic construct

SEQ ID NO: 195 - protein, 120 aa, Artificial Sequence
  Synthetic construct
EVQLVESGPGLVKPSETLSLTCTVSGFSLTRFGVHWVRQPPGKGLEWLGVIWRGGSTDYNPAFMSRLTISKDNSKNQVSLKLSSVTAADTAVYYCSNHYYGSSDYALDNWGQGTLVTVSS

SEQ ID NO: 196 - protein, 107 aa, Artificial Sequence; identical to SEQ ID NO: 83
  Synthetic construct

SEQ ID NO: 197 - protein, 120 aa, Artificial Sequence
  Synthetic construct
EVQLVESGPGLVKPSETLSLTCTVSGFSLTRFGVHWVRQPPGKGLEWLGVIWRGGSTDYNAAFGSRLTISKDNSKNQVSLKLSSVTAADTAVYYCSNHYYGSSDYALDNWGQGTLVTVSS

SEQ ID NO: 198 - protein, 107 aa, Artificial Sequence; identical to SEQ ID NO: 83
  Synthetic construct

SEQ ID NO: 199 - protein, 120 aa, Artificial Sequence
  Synthetic construct
EVQLVESGPGLVKPSETLSLTCTVSGFSLTRFGVHWVRQPPGKGLEWLGVIWRGGSTDYNAAFMDRLTISKDNSKNQVSLKLSSVTAADTAVYYCSNHYYGSSDYALDNWGQGTLVTVSS

SEQ ID NO: 200 - protein, 107 aa, Artificial Sequence; identical to SEQ ID NO: 83
  Synthetic construct

SEQ ID NO: 201 - protein, 120 aa, Artificial Sequence
  Synthetic construct
EVQLVESGPGLVKPSETLSLTCTVSGFSLTRFGVHWVRQPPGKGLEWLGVIWRGGSTDYNAAFMPRLTISKDNSKNQVSLKLSSVTAADTAVYYCSNHYYGSSDYALDNWGQGTLVTVSS

SEQ ID NO: 202 - protein, 107 aa, Artificial Sequence; identical to SEQ ID NO: 83
  Synthetic construct

SEQ ID NO: 203 - protein, 120 aa, Artificial Sequence
  Synthetic construct
EVQLVESGPGLVKPSETLSLTCTVSGFSLTRFGVHWVRQPPGKGLEWLGVIWRGGSTDYNAAFMSRLTISKDNSKNQVSLMLSSVTAADTAVYYCSNHYYGSSDYALDNWGQGTLVTVSS

SEQ ID NO: 204 - protein, 107 aa, Artificial Sequence; identical to SEQ ID NO: 83
  Synthetic construct

SEQ ID NO: 205 - protein, 120 aa, Artificial Sequence
  Synthetic construct
EVQLVESGPGLVKPSETLSLTCTVSGFSLTRFGVHWVRQPPGKGLEWLGVIWRGGSTDYNAAFMSRLTISKDNSKNQVSLKLSDVTAADTAVYYCSNHYYGSSDYALDNWGQGTLVTVSS

SEQ ID NO: 206 - protein, 107 aa, Artificial Sequence; identical to SEQ ID NO: 83
  Synthetic construct

SEQ ID NO: 207 - protein, 120 aa, Artificial Sequence
  Synthetic construct
EVQLVESGPGLVKPSETLSLTCTVSGFSLTRFGVHWVRQPPGKGLEWLGVIWRGGSTDYNAAFMSRLTISKDNSKNQVSLKLSSVTAADTAVYYCSNHYYGSPDYALDNWGQGTLVTVSS

SEQ ID NO: 208 - protein, 107 aa, Artificial Sequence; identical to SEQ ID NO: 83
  Synthetic construct

SEQ ID NO: 209 - protein, 120 aa, Artificial Sequence; identical to SEQ ID NO: 102
  Synthetic construct

SEQ ID NO: 210 - protein, 107 aa, Artificial Sequence
  Synthetic construct
DIQMTQSPSSLSASVGDRVTITCKASQDVSNLVVWFQQKPGKSPKLLIYSGSYRYSGVPSRFSGSGSGTDFTLTISSLQPEDFATYYCQQHYSPPYTFGQGTKVEIK

SEQ ID NO: 211 - protein, 120 aa, Artificial Sequence
  Synthetic construct
EVQLVESGPGLVKPSETLSLTCTVSGFSTTRFGVHWVRQPPGKGLEWLGVIWRGGSTDYNAAFVSRLTISKDNSKNQVSLKLSSVTAADTAVYYCSNHYYGSSDYALDNWGQGTLVTVSS

SEQ ID NO: 212 - protein, 107 aa, Artificial Sequence; identical to SEQ ID NO: 210
  Synthetic construct

SEQ ID NO: 213 - protein, 120 aa, Artificial Sequence
  Synthetic construct
EVQLVESGPGLVKPSETLSLTCTVSGFSLTRFGVHWVRQPPGKGLEWLGVIWRGGSTDYNAAFVSRLTISKDNSKNQVSLKLSSVTAADTAVYYCSNHYYGSPDYALDNWGQGTLVTVSS

SEQ ID NO: 214 - protein, 107 aa, Artificial Sequence; identical to SEQ ID NO: 210
  Synthetic construct

SEQ ID NO: 215 - protein, 975 aa, Macaca fascicularis
MLLWVILLVLAPVSGQFVRTYKSHFLQPPWTTVFRGERVNLTCKGFGFYSSQKTKWYYRHLGKEISRETQKNTLEVQESGEYRCQAQGSPLSSPVSLDFSSASLILQAPLSVFEGDSVVLRCRAKAEVTLKTTIYKNENVLAFLNKSTDFHISHASLKDNGAYRCTGYKETCCLVSSNTVKIQVQESFTRPVLRVSSFQPISGSPVTLTCETQLSLERSDVPLQFCFFRNDQMLGSGCSLSPKFRITAMWSKDSGSYWCKAATMCYDTTSNSLRSWIQVLIPASHPVLTLSPEKALNFEGTKVKLHCETQEDSLRTLYKFYHDGVPLRYKSVRCEKGASISFSLTTEHSGNYYCTADNGHGAKPSEAVSLSVTVPVSRPVLTLSSAEDLISEGAKLTLHCEAQRGSLPIVYQFHHENASLGNRSAHSAGGVAISFSLTADHSGNYYCTANNGFGPQRSEAVSLSITVPVSRPVLTLSSAEALTFEGATVTLYCEVQRGSPRILYQFYHEDVPLGSNSTPSVGKVSFSFSLTAAHSGNYYCTADNGFGPQRSEAVSLFVTVPVSRPILTLRVPRAQAVVGDLLELRCEALRGSPPIMYWFYHEDVTLGSSSVPSGGEASFNLSLTAEHSGNYSCEANNGLVAQHSDTISLSVIVPVSRPILTFRAPRAQAVVGDLLELHCEALRGSSPILYWFYHEDVTLGKISAPSGGGAYFNLSLTTEHSGIYSCEADNGLEAQRSEMVTLKVAVPVSRPVLTLRAPRAQVAVGDLLELHCEALRGSPLILYQFYHEDVTLGNSSALSGGAFFNLSLTAEHGNYSCEADNGLGAQRSETVTLYLTGLTENRSGPVATGVTGGLLSLAGLAAVALLLYCWLSRKAGREPASDPCRSPSDLDSQEPTYHNVPAWEELQPVYSNVNPRGENVVYSEVRIIREKKKHAVASNPRHLRNKGSCIIYSEVKVASTPASRCLFLASSAPHR